European Patent Specification EP 3 583 209 B1, published December 4, 2024. Title: HIGH-FIDELITY CAS9 VARIANTS AND APPLICATIONS THEREOF. Applicant: Università degli Studi di Trento. The sequence listing filed with the application follows.

SEQUENCE LISTING (138 sequences)

SEQ ID NO: 1 - protein, 1368 aa, Streptococcus pyogenes [sequence omitted]

SEQ ID NO: 2 - DNA, 4107 bp, Streptococcus pyogenes M1 GAS
  ref <308>: NC_002737.2
  ref <309>: 2016-08-03
  ref <313>: (854751)..(858857)
atggataagaaatactcaataggcttagatatcggcacaaatagcgtcggatgggcggtgatcactgatgaatataaggttccgtctaaaaagttcaaggttctgggaaatacagaccgccacagtatcaaaaaaaatcttataggggctcttttatttgacagtggagagacagcggaagcgactcgtctcaaacggacagctcgtagaaggtatacacgtcggaagaatcgtatttgttatctacaggagattttttcaaatgagatggcgaaagtagatgatagtttctttcatcgacttgaagagtcttttttggtggaagaagacaagaagcatgaacgtcatcctatttttggaaatatagtagatgaagttgcttatcatgagaaatatccaactatctatcatctgcgaaaaaaattggtagattctactgataaagcggatttgcgcttaatctatttggccttagcgcatatgattaagtttcgtggtcattttttgattgagggagatttaaatcctgataatagtgatgtggacaaactatttatccagttggtacaaacctacaatcaattatttgaagaaaaccctattaacgcaagtggagtagatgctaaagcgattctttctgcacgattgagtaaatcaagacgattagaaaatctcattgctcagctccccggtgagaagaaaaatggcttatttgggaatctcattgctttgtcattgggtttgacccctaattttaaatcaaattttgatttggcagaagatgctaaattacagctttcaaaagatacttacgatgatgatttagataatttattggcgcaaattggagatcaatatgctgatttgtttttggcagctaagaatttatcagatgctattttactttcagatatcctaagagtaaatactgaaataactaaggctcccctatcagcttcaatgattaaacgctacgatgaacatcatcaagacttgactcttttaaaagctttagttcgacaacaacttccagaaaagtataaagaaatcttttttgatcaatcaaaaaacggatatgcaggttatattgatgggggagctagccaagaagaattttataaatttatcaaaccaattttagaaaaaatggatggtactgaggaattattggtgaaactaaatcgtgaagatttgctgcgcaagcaacggacctttgacaacggctctattccccatcaaattcacttgggtgagctgcatgctattttgagaagacaagaagacttttatccatttttaaaagacaatcgtgagaagattgaaaaaatcttgacttttcgaattccttattatgttggtccattggcgcgtggcaatagtcgttttgcatggatgactcggaagtctgaagaaacaattaccccatggaattttgaagaagttgtcgataaaggtgcttcagctcaatcatttattgaacgcatgacaaactttgataaaaatcttccaaatgaaaaagtactaccaaaacatagtttgctttatgagtattttacggtttataacgaattgacaaaggtcaaatatgttactgaaggaatgcgaaaaccagcatttctttcaggtgaacagaagaaagccattgttgatttactcttcaaaacaaatcgaaaagtaaccgttaagcaattaaaagaagattatttcaaaaaaatagaatgttttgatagtgttgaaatttcaggagttgaagatagatttaatgcttcattaggtacctaccatgatttgctaaaaattattaaagataaagattttttggataatgaagaaaatgaagatatcttagaggatattgttttaacattgaccttatttgaagatagggagatgattgaggaaagacttaaaacatatgctcacctctttgatgataaggtgatgaaacagcttaaacgtcgccgttatactggttggggacgtttgtctcgaaaattgattaatggtattagggataagcaatctggcaaaacaatattagattttttgaaatcagatggttttgccaatcgcaattttatgcagctgatccatgatgatagtttgacatttaaagaagacattcaaaaagcacaagtgtctggacaaggcgatagtttacatgaacatattgcaaatttagctggtagccctgctattaaaaaaggtattttacagactgtaaaagttgttgatgaattggtcaaagtaatggggcggcataagccagaaaatatcgttattgaaatggcacgtgaaaatcagacaactcaaaagggccagaaaaattcgcgagagcgtatgaaacgaatcgaagaaggtatcaaagaattaggaagtcagattcttaaagagcatcctgttgaaaatactcaattgcaaaatgaaaagctctatctctattatctccaaaatggaagagacatgtatgtggaccaagaattagatattaatcgtttaagtgattatgatgtcgatcacattgttccacaaagtttccttaaagacgattcaatagacaataaggtcttaacgcgttctgataaaaatcgtggtaaatcggataacgttccaagtgaagaagtagtcaaaaagatgaaaaactattggagacaacttctaaacgccaagttaatcactcaacgtaagtttgataatttaacgaaagctgaacgtggaggtttgagtgaacttgataaagctggttttatcaaacgccaattggttgaaactcgccaaatcactaagcatgtggcacaaattttggatagtcgcatgaatactaaatacgatgaaaatgataaacttattcgagaggttaaagtgattaccttaaaatctaaattagtttctgacttccgaaaagatttccaattctataaagtacgtgagattaacaattaccatcatgcccatgatgcgtatctaaatgccgtcgttggaactgctttgattaagaaatatccaaaacttgaatcggagtttgtctatggtgattataaagtttatgatgttcgtaaaatgattgctaagtctgagcaagaaataggcaaagcaaccgcaaaatatttcttttactctaatatcatgaacttcttcaaaacagaaattacacttgcaaatggagagattcgcaaacgccctctaatcgaaactaatggggaaactggagaaattgtctgggataaagggcgagattttgccacagtgcgcaaagtattgtccatgccccaagtcaatattgtcaagaaaacagaagtacagacaggcggattctccaaggagtcaattttaccaaaaagaaattcggacaagcttattgctcgtaaaaaagactgggatccaaaaaaatatggtggttttgatagtccaacggtagcttattcagtcctagtggttgctaaggtggaaaaagggaaatcgaagaagttaaaatccgttaaagagttactagggatcacaattatggaaagaagttcctttgaaaaaaatccgattgactttttagaagctaaaggatataaggaagttaaaaaagacttaatcattaaactacctaaatatagtctttttgagttagaaaacggtcgtaaacggatgctggctagtgccggagaattacaaaaaggaaatgagctggctctgccaagcaaatatgtgaattttttatatttagctagtcattatgaaaagttgaagggtagtccagaagataacgaacaaaaacaattgtttgtggagcagcataagcattatttagatgagattattgagcaaatcagtgaattttctaagcgtgttattttagcagatgccaatttagataaagttcttagtgcatataacaaacatagagacaaaccaatacgtgaacaagcagaaaatattattcatttatttacgttgacgaatcttggagctcccgctgcttttaaatattttgatacaacaattgatcgtaaacgatatacgtctacaaaagaagttttagatgccactcttatccatcaatccatcactggtctttatgaaacacgcattgatttgagtcagctaggaggtgactga

SEQ ID NO: 3 - DNA, 4107 bp, Streptococcus pyogenes
atggacaagaagtacagcatcggcctggacatcggcaccaactctgtgggctgggccgtgatcaccgacgagtacaaggtgcccagcaagaaattcaaggtgctgggcaacaccgaccggcacagcatcaagaagaacctgatcggagccctgctgttcgacagcggcgaaacagccgaggccacccggctgaagagaaccgccagaagaagatacaccagacggaagaaccggatctgctatctgcaagagatcttcagcaacgagatggccaaggtggacgacagcttcttccacagactggaagagtccttcctggtggaagaggataagaagcacgagcggcaccccatcttcggcaacatcgtggacgaggtggcctaccacgagaagtaccccaccatctaccacctgagaaagaaactggtggacagcaccgacaaggccgacctgcggctgatctatctggccctggcccacatgatcaagttccggggccacttcctgatcgagggcgacctgaaccccgacaacagcgacgtggacaagctgttcatccagctggtgcagacctacaaccagctgttcgaggaaaaccccatcaacgccagcggcgtggacgccaaggccatcctgtctgccagactgagcaagagcagacggctggaaaatctgatcgcccagctgcccggcgagaagaagaatggcctgttcggaaacctgattgccctgagcctgggcctgacccccaacttcaagagcaacttcgacctggccgaggatgccaaactgcagctgagcaaggacacctacgacgacgacctggacaacctgctggcccagatcggcgaccagtacgccgacctgtttctggccgccaagaacctgtccgacgccatcctgctgagcgacatcctgagagtgaacaccgagatcaccaaggcccccctgagcgcctctatgatcaagagatacgacgagcaccaccaggacctgaccctgctgaaagctctcgtgcggcagcagctgcctgagaagtacaaagagattttcttcgaccagagcaagaacggctacgccggctacattgacggcggagccagccaggaagagttctacaagttcatcaagcccatcctggaaaagatggacggcaccgaggaactgctcgtgaagctgaacagagaggacctgctgcggaagcagcggaccttcgacaacggcagcatcccccaccagatccacctgggagagctgcacgccattctgcggcggcaggaagatttttacccattcctgaaggacaaccgggaaaagatcgagaagatcctgaccttccgcatcccctactacgtgggccctctggccaggggaaacagcagattcgcctggatgaccagaaagagcgaggaaaccatcaccccctggaacttcgaggaagtggtggacaagggcgcttccgcccagagcttcatcgagcggatgaccaacttcgataagaacctgcccaacgagaaggtgctgcccaagcacagcctgctgtacgagtacttcaccgtgtataacgagctgaccaaagtgaaatacgtgaccgagggaatgagaaagcccgccttcctgagcggcgagcagaaaaaggccatcgtggacctgctgttcaagaccaaccggaaagtgaccgtgaagcagctgaaagaggactacttcaagaaaatcgagtgcttcgactccgtggaaatctccggcgtggaagatcggttcaacgcctccctgggcacataccacgatctgctgaaaattatcaaggacaaggacttcctggacaatgaggaaaacgaggacattctggaagatatcgtgctgaccctgacactgtttgaggacagagagatgatcgaggaacggctgaaaacctatgcccacctgttcgacgacaaagtgatgaagcagctgaagcggcggagatacaccggctggggcaggctgagccggaagctgatcaacggcatccgggacaagcagtccggcaagacaatcctggatttcctgaagtccgacggcttcgccaacagaaacttcatgcagctgatccacgacgacagcctgacctttaaagaggacatccagaaagcccaggtgtccggccagggcgatagcctgcacgagcacattgccaatctggccggcagccccgccattaagaagggcatcctgcagacagtgaaggtggtggacgagctcgtgaaagtgatgggccggcacaagcccgagaacatcgtgatcgaaatggccagagagaaccagaccacccagaagggacagaagaacagccgcgagagaatgaagcggatcgaagagggcatcaaagagctgggcagccagatcctgaaagaacaccccgtggaaaacacccagctgcagaacgagaagctgtacctgtactacctgcagaatgggcgggatatgtacgtggaccaggaactggacatcaaccggctgtccgactacgatgtggaccatatcgtgcctcagagctttctgaaggacgactccatcgacaacaaggtgctgaccagaagcgacaagaaccggggcaagagcgacaacgtgccctccgaagaggtcgtgaagaagatgaagaactactggcggcagctgctgaacgccaagctgattacccagagaaagttcgacaatctgaccaaggccgagagaggcggcctgagcgaactggataaggccggcttcatcaagagacagctggtggaaacccggcagatcacaaagcacgtggcacagatcctggactcccggatgaacactaagtacgacgagaatgacaagctgatccgggaagtgaaagtgatcaccctgaagtccaagctggtgtccgatttccggaaggatttccagttttacaaagtgcgcgagatcaacaactaccaccacgcccacgacgcctacctgaacgccgtcgtgggaaccgccctgatcaaaaagtaccctaagctggaaagcgagttcgtgtacggcgactacaaggtgtacgacgtgcggaagatgatcgccaagagcgagcaggaaatcggcaaggctaccgccaagtacttcttctacagcaacatcatgaactttttcaagaccgagattaccctggccaacggcgagatccggaagcggcctctgatcgagacaaacggcgaaaccggggagatcgtgtgggataagggccgggattttgccaccgtgcggaaagtgctgagcatgccccaagtgaatatcgtgaaaaagaccgaggtgcagacaggcggcttcagcaaagagtctatcctgcccaagaggaacagcgataagctgatcgccagaaagaaggactgggaccctaagaagtacggcggcttcgacagccccaccgtggcctattctgtgctggtggtggccaaagtggaaaagggcaagtccaagaaactgaagagtgtgaaagagctgctggggatcaccatcatggaaagaagcagcttcgagaagaatcccatcgactttctggaagccaagggctacaaagaagtgaaaaaggacctgatcatcaagctgcctaagtactccctgttcgagctggaaaacggccggaagagaatgctggcctctgccggcgaactgcagaagggaaacgaactggccctgccctccaaatatgtgaacttcctgtacctggccagccactatgagaagctgaagggctcccccgaggataatgagcagaaacagctgtttgtggaacagcacaagcactacctggacgagatcatcgagcagatcagcgagttctccaagagagtgatcctggccgacgctaatctggacaaagtgctgtccgcctacaacaagcaccgggataagcccatcagagagcaggccgagaatatcatccacctgtttaccctgaccaatctgggagcccctgccgccttcaagtactttgacaccaccatcgaccggaagaggtacaccagcaccaaagaggtgctggacgccaccctgatccaccagagcatcaccggcctgtacgagacacggatcgacctgtctcagctgggaggcgactaa

SEQ ID NO: 4 - DNA, 35 bp, Artificial Sequence
  Synthetic construct
ccagaaagcacaagttgctagccagggggacagtc

SEQ ID NO: 5 - DNA, 35 bp, Artificial Sequence
  Synthetic construct
gactgtccccctggctagcaacttgtgctttctgg

SEQ ID NO: 6 - DNA, 32 bp, Artificial Sequence
  Synthetic construct
cagcgcactttcgaccatggaagcatccccca

SEQ ID NO: 7 - DNA, 32 bp, Artificial Sequence
  Synthetic construct
tgggggatgcttccatggtcgaaagtgcgctg

SEQ ID NO: 8 - DNA, 20 bp, Serratia phage SM9-3Y, 9162-9181
  ref <308>: KX778611.1
  ref <309>: 2017-01-17
  ref <313>: (9162)..(9181)
aattaaccctcactaaaggg

SEQ ID NO: 9 - DNA, 20 bp, Escherichia coli strain Y5, 1391073-1391092
  ref <308>: CP013483.1
  ref <309>: 2016-11-01
  ref <313>: (1391073)..(1391092)
taatacgactcactataggg

SEQ ID NO: 10 - DNA, 42 bp, Artificial Sequence
  Synthetic construct
ctcgtgaccaccctgacctagttttagagctagaaatagcaa

SEQ ID NO: 11 - DNA, 41 bp, Artificial Sequence
  Synthetic construct
taggtcagggtggtcacgaggatcatttatctttcactgcg

SEQ ID NO: 12 - DNA, 19 bp, Artificial Sequence
  Synthetic construct
acgtgggccctctggccag

SEQ ID NO: 13 - DNA, 31 bp, Artificial Sequence
  Synthetic construct
tacgctagctccctttttcttttttgcctgg

SEQ ID NO: 14 - DNA, 26 bp, Artificial Sequence
  Synthetic construct
attagggccccctggcccgagggaac

SEQ ID NO: 15 - DNA, 31 bp, Artificial Sequence
  Synthetic construct
taatactagtgactttcctcttcttcttggg

SEQ ID NO: 16 - DNA, 19 bp, Saccharomyces cerevisiae YJM1549 chromosome IV
  ref <308>: CP004747.2
  ref <309>: 2016-09-16
  ref <313>: (453079)..(453097)
ccaagagggagggcattgg

SEQ ID NO: 17 - DNA, 55 bp, Artificial Sequence
  Synthetic construct
tgcggtaccgtaggtcagggtggtcacgagttagaggaactcttggtattcttgc

SEQ ID NO: 18 - DNA, 33 bp, Artificial Sequence
  Synthetic construct
ttaggtaccgtaatcaacctaaggaggatgttt

SEQ ID NO: 19 - DNA, 22 bp, Saccharomyces cerevisiae YJM1549 chromosome IV
  ref <308>: CP004747.2
  ref <309>: 2016-09-16
  ref <313>: (453875)..(453896)
tgcttgcttttcaaaaggcctg

SEQ ID NO: 20 - DNA, 26 bp, Saccharomyces cerevisiae YJM1574 chromosome XV
  ref <308>: CP005677.2
  ref <309>: 2016-11-22
  ref <313>: (548437)..(548462)
tgcctagtttcatgaaattttaaagc

SEQ ID NO: 21 - DNA, 53 bp, Artificial Sequence
  Synthetic construct
ccaggatccggaggtcagggtggtcacgagttagacgcaagcatcaatggtat

SEQ ID NO: 22 - DNA, 53 bp, Artificial Sequence
  Synthetic construct
ccaggatccgtaggtaagggtggtcacgagttagacgcaagcatcaatggtat

SEQ ID NO: 23 - DNA, 53 bp, Artificial Sequence
  Synthetic construct
ccaggatccgtaggtcagggcggtcacgagttagacgcaagcatcaatggtat

SEQ ID NO: 24 - DNA, 53 bp, Artificial Sequence
  Synthetic construct
ccaggatccgtaggtcagggtggtaacgagttagacgcaagcatcaatggtat

SEQ ID NO: 25 - DNA, 33 bp, Artificial Sequence
  Synthetic construct
attaggatcctggtgtggaaatgttctatttag

SEQ ID NO: 26 - DNA, 27 bp, Saccharomyces cerevisiae YJM1574 chromosome XV
  ref <308>: CP005677.2
  ref <309>: 2016-11-22
  ref <313>: (546227)..(546253)
gtaatcataacaaagcctaaaaaatag

SEQ ID NO: 27 - DNA, 88 bp, Artificial Sequence
  Synthetic construct
tattgagcacgtgagtatacgtgattaagcacacaaaggcagcttggagttagggataacagggtaatttggatggacgcaaagaagt

SEQ ID NO: 28 - DNA, 70 bp, Artificial Sequence
  Synthetic construct
tgcaggcaagtgcacaaacaatacttaaataaatactactcagtaataacttcgtacgctgcaggtcgac

SEQ ID NO: 29 - DNA, 88 bp, Artificial Sequence
  Synthetic construct
cctactataacaatcaagaaaaacaagaaaatcggacaaaacaatcaagttagggataacagggtaatttggatggacgcaaagaagt

SEQ ID NO: 30 - DNA, 70 bp, Artificial Sequence
  Synthetic construct
atatcattttataattatttgctgtacaagtatatcaataaacttatatattcgtacgctgcaggtcgac

SEQ ID NO: 31 - DNA, 23 bp, Artificial Sequence
  Synthetic construct
ctcgtgaccaccctgacctacgg

SEQ ID NO: 32 - DNA, 23 bp, Artificial Sequence
  Synthetic construct
ctcgtgaccaccctgacctccgg

SEQ ID NO: 33 - DNA, 23 bp, Artificial Sequence
  Synthetic construct
ctcgtgaccacccttacctacgg

SEQ ID NO: 34 - DNA, 23 bp, Artificial Sequence
  Synthetic construct
ctcgtgaccgccctgacctacgg

SEQ ID NO: 35 - DNA, 23 bp, Artificial Sequence
  Synthetic construct
ctcgttaccaccctgacctacgg

SEQ ID NO: 36 - DNA, 50 bp, Artificial Sequence
  Synthetic construct
gtctaaaaatggctacgccggatacattgacggcggagcaagccaggagg

SEQ ID NO: 37 - DNA, 50 bp, Artificial Sequence
  Synthetic construct
tctcgggccatctcgataacgatattctcgggcttatgccttcccattac

SEQ ID NO: 38 - DNA, 20 bp, Artificial Sequence
  Synthetic construct
gggcacgggcagcttgccgg

SEQ ID NO: 39 - DNA, 20 bp, Artificial Sequence
  Synthetic construct
gggcacccgcagcttgccgg

SEQ ID NO: 40 - DNA, 20 bp, Artificial Sequence
  Synthetic construct
gcccacgggcagcttgccgg

SEQ ID NO: 41 - DNA, 20 bp, Artificial Sequence
  Synthetic construct
ggccacgggcagcttgccgg

SEQ ID NO: 42 - DNA, 20 bp, Artificial Sequence
  Synthetic construct
gtcgccctcgaacttcacct

SEQ ID NO: 43 - DNA, 20 bp, Artificial Sequence
  Synthetic construct
gaagggcatcgacttcaagg

SEQ ID NO: 44 - DNA, 20 bp, Artificial Sequence
  Synthetic construct
gctgaagcactgcacgccgt

SEQ ID NO: 45 - DNA, 20 bp, Artificial Sequence
  Synthetic construct
gaccaggatgggcaccaccc

SEQ ID NO: 46 - DNA, 20 bp, Artificial Sequence
  Synthetic construct
gaagttcgagggcgacaccc

SEQ ID NO: 47 - DNA, 19 bp, Artificial Sequence
  Synthetic construct
ggcacgggcagcttgccgg

SEQ ID NO: 48 - DNA, 18 bp, Artificial Sequence
  Synthetic construct
ggcaagctgcccgtgccc

SEQ ID NO: 49 - DNA, 17 bp, Artificial Sequence
  Synthetic construct
gtgaccaccctgaccta

SEQ ID NO: 50 - DNA, 20 bp, Artificial Sequence
  Synthetic construct
gtgatagagaacgtatgtcg

SEQ ID NO: 51 - DNA, 21 bp, Artificial Sequence
  Synthetic construct
ggtgatagagaacgtatgtcg

SEQ ID NO: 52 - DNA, 20 bp, Artificial Sequence
  Synthetic construct
gtgatagagaacgtctgtcg

SEQ ID NO: 53 - DNA, 20 bp, Artificial Sequence
  Synthetic construct
gtgatactgaacgtatgtcg

SEQ ID NO: 54 - DNA, 20 bp, Artificial Sequence
  Synthetic construct
gacatagagaacgtatgtcg

SEQ ID NO: 55 - DNA, 33 bp, Artificial Sequence
  Synthetic construct
tcgtcggcagcgtcagatgtgtataagagacag

SEQ ID NO: 56 - DNA, 34 bp, Artificial Sequence
  Synthetic construct
gtctcgtgggctcggagatgtgtataagagacag

SEQ ID NO: 57 - DNA, 23 bp, Homo sapiens, chr2:72933853-72933875
gagtccgagcagaagaagaaggg

SEQ ID NO: 58 - DNA, 23 bp, Homo sapiens, chr2:72933807-72933829
ccggaggacaaagtacaaacggc

SEQ ID NO: 59 - DNA, 21 bp, Homo sapiens, chr2:72933973-72933993
aagcagcactctgccctcgtg

SEQ ID NO: 60 - DNA, 23 bp, Homo sapiens, chr5:45358959-45358981
gagttagagcagaagaagaaagg

SEQ ID NO: 61 - DNA, 25 bp, Homo sapiens, chr5:45359021-45359045
cttttataccatcttggggttacag

SEQ ID NO: 62 - DNA, 27 bp, Homo sapiens, chr5:45358831-45358857
ctaggaaagattaacagagagtctgac

SEQ ID NO: 63 - DNA, 23 bp, Homo sapiens, chr15:43817549-43817571
gagtctaagcagaagaagaagag

SEQ ID NO: 64 - DNA, 24 bp, Homo sapiens, chr15:43817490-43817513
caatgtgcttcaacccatcacggc

SEQ ID NO: 65 - DNA, 27 bp, Homo sapiens, chr15:43817671-43817697
cctctacttcattgtactcaaggtaag

SEQ ID NO: 66 - DNA, 23 bp, Homo sapiens, chr5:9227034-9227056
aagtctgagcacaagaagaatgg

SEQ ID NO: 67 - DNA, 24 bp, Homo sapiens, chr5:9226951-9226974
tagttctgacattcctcctgaggg

SEQ ID NO: 68 - DNA, 29 bp, Homo sapiens, chr5:9227136-9227164
ctctgttgttattttttggtcaatatctg

SEQ ID NO: 69 - DNA, 23 bp, Homo sapiens, chr8:127788996-127789018
gagtcctagcaggagaagaagag

SEQ ID NO: 70 - DNA, 21 bp, Homo sapiens, chr8:127788953-127788973
aaagcctggaggctgccaggt

SEQ ID NO: 71 - DNA, 24 bp, Homo sapiens, chr8:127789131-127789154
atctagctgtcctgtctcattggc

SEQ ID NO: 72 - DNA, 23 bp, Homo sapiens, chr2:218980334-218980356
gaggccgagcagaagaaagacgg

SEQ ID NO: 73 - DNA, 17 bp, Homo sapiens, chr2:10350-10366
  ref <308>: NG_023323.1
  ref <309>: 2016-10-07
  ref <313>: (10350)..(10366)
caggagccgggtgggag

SEQ ID NO: 74 - DNA, 21 bp, Homo sapiens, chr2:218980463-218980483
cctcagccttccctcagccac

SEQ ID NO: 75 - DNA, 23 bp, Homo sapiens, chr6:43769717-43769739
ggtgagtgagtgtgtgcgtgtgg

SEQ ID NO: 76 - DNA, 21 bp, Homo sapiens, chr6:43769662-43769682
ctgggtgaatggagcgagcag

SEQ ID NO: 77 - DNA, 20 bp, Homo sapiens, chr6:43769824-43769843
ggaaggcggagagccggaca

SEQ ID NO: 78 - DNA, 23 bp, Homo sapiens, chr14:65102435-65102457
agtgagtgagtgtgtgtgtgggg

SEQ ID NO: 79 - DNA, 21 bp, Homo sapiens, chr14:65102393-65102413
gaaggggagggggaagtcacc

SEQ ID NO: 80 - DNA, 20 bp, Homo sapiens, chr14:65102527-65102546
cgtgcgtgccgccgttgatc

SEQ ID NO: 81 - DNA, 23 bp, Homo sapiens, chr5:116098962-116098984
tgtgggtgagtgtgtgcgtgagg

SEQ ID NO: 82 - DNA, 23 bp, Homo sapiens, chr5:116098932-116098954
tctgtcaccacacagttaccacc

SEQ ID NO: 83 - DNA, 24 bp, Homo sapiens, chr5:116099133-116099156
gtagttgcctggggatggggtatg

SEQ ID NO: 84 - DNA, 23 bp, Homo sapiens, chr22:37266777-37266799
gctgagtgagtgtatgcgtgtgg

SEQ ID NO: 85 - DNA, 25 bp, Homo sapiens, chr22:37266726-37266750
cacctggcccatttctcctttgagg

SEQ ID NO: 86 - DNA, 24 bp, Homo sapiens, chr22:37266856-37266879
tggggacagcatgtgcaagccaca

SEQ ID NO: 87 - DNA, 23 bp, Homo sapiens, chr14:29676-29698
  ref <308>: KI270846.1
  ref <309>: 2017-01-06
  ref <313>: (29676)..(29698)
ggtgagtgagtgtgtgtgtgagg

SEQ ID NO: 88 - DNA, 21 bp, Homo sapiens, chr14:29625-29645
  ref <308>: KI270846.1
  ref <309>: 2017-01-06
  ref <313>: (29625)..(29645)
ggacccctctgacagactgca

SEQ ID NO: 89 - DNA, 23 bp, Homo sapiens, chr14:29760-29782
  ref <308>: KI270846.1
  ref <309>: 2017-01-06
  ref <313>: (29760)..(29782)
cacacaccctcacataccctcac

SEQ ID NO: 90 - DNA, 23 bp, Homo sapiens, chr5:90145146-90145168
agagagtgagtgtgtgcatgagg

SEQ ID NO: 91 - DNA, 27 bp, Homo sapiens, chr5:90145191-90145217
ggaagaatgcaaaggagaagcaagtac

SEQ ID NO: 92 - DNA, 24 bp, Homo sapiens, chr5:90145038-90145061
gacctggtgggagttgattggatc

SEQ ID NO: 93 - DNA, 23 bp, Homo sapiens, chr20:20197634-20197656
agtgtgtgagtgtgtgcgtgtgg

SEQ ID NO: 94 - DNA, 27 bp, Homo sapiens, chr20:20197688-20197714
ccttgggaatctatcttgaataggcct

SEQ ID NO: 95 - DNA, 22 bp, Homo sapiens, chr20:20197546-20197567
gacaccccacacactctcatgc

SEQ ID NO: 96 - DNA, 23 bp, Homo sapiens, chr14:61612049-61612071
tgtgagtaagtgtgtgtgtgtgg

SEQ ID NO: 97 - DNA, 24 bp, Homo sapiens, chr14:61612099-61612122
cctaagctgtatgtgagtccctga

SEQ ID NO: 98 - DNA, 29 bp, Homo sapiens, chr14:61611941-61611969
ctgttttgctaagagatgattagatggtc

SEQ ID NO: 99 - DNA, 23 bp, Homo sapiens, chr10:97000825-97000847
gttgagtgaatgtgtgcgtgagg

SEQ ID NO: 100 - DNA, 21 bp, Homo sapiens, chr10:97000874-97000894
gccctctccggaagtgccttg

SEQ ID NO: 101 - DNA, 24 bp, Homo sapiens, chr10:97000734-97000757
gaagggttggtttggaaggctgtc

SEQ ID NO: 102 - DNA, 23 bp, Homo sapiens, chr11:69083658-69083680
ggtgagtgagtgcgtgcgggtgg

SEQ ID NO: 103 - DNA, 24 bp, Homo sapiens, chr11:69083595-69083618
ccacaggaatttgaagtccgtgct

SEQ ID NO: 104 - DNA, 22 bp, Homo sapiens, chr11:69083735-69083756
ccccacgtccacccatacacac

SEQ ID NO: 105 - DNA, 23 bp, Homo sapiens, chr14:73886777-73886799
agcgagtgggtgtgtgcgtgggg

SEQ ID NO: 106 - DNA, 21 bp, Homo sapiens, chr14:73886731-73886751
gacgtctgggtcccgagcagt

SEQ ID NO: 107 - DNA, 19 bp, Homo sapiens, chr14:73886873-73886891
ggccgtcagtcggtcccga

SEQ ID NO: 108 - DNA, 23 bp, Homo sapiens, chr16:79982417-79982439
tgtgagtgagtgtgtgcgtgtga

SEQ ID NO: 109 - DNA, 25 bp, Homo sapiens, chr16:79982476-79982500
ggagggttgaactgtgacagaactg

SEQ ID NO: 110 - DNA, 26 bp, Homo sapiens, chr16:79982303-79982328
tgagtatgtgtgagtgagagtgtgca

SEQ ID NO: 111 - DNA, 23 bp, Homo sapiens, chr19:40055954-40055976
actgtgtgagtgtgtgcgtgagg

SEQ ID NO: 112 - DNA, 21 bp, Homo sapiens, chr19:40056024-40056044
gatccttaggcgtgcgtgtgc

SEQ ID NO: 113 - DNA, 21 bp, Homo sapiens, chr19:40055878-40055898
caccggcacagtgacactcac

SEQ ID NO: 114 - DNA, 23 bp, Homo sapiens, chr5:29367266-29367288
tgtgagtgagtgtgtgtatgggg

SEQ ID NO: 115 - DNA, 24 bp, Homo sapiens, chr5:29367302-29367325
agaccttcaatgtggatgtgcgtg

SEQ ID NO: 116 - DNA, 29 bp, Homo sapiens, chr5:29367042-29367070
catagagtgtagcagatttccataacttc

SEQ ID NO: 117 - DNA, 22 bp, Homo sapiens, chr6:43769231-43769252
gcatacgtgggctccaacaggt

SEQ ID NO: 118 - DNA, 22 bp, Homo sapiens, chr6:43770011-43770032
ccgcaatgaaggggaagctcga

SEQ ID NO: 119 - DNA, 23 bp, Homo sapiens, chr15:84621797-84621819
gtgcggcaagagcttcagccggg

SEQ ID NO: 120 - DNA, 21 bp, Homo sapiens, chr15:84621375-84621395
gactgtgggcagaggttcagc

SEQ ID NO: 121 - DNA, 24 bp, Homo sapiens, chr15:84622203-84622226
tgtatacgggacttgactcagacc

SEQ ID NO: 122 - DNA, 23 bp, Homo sapiens, chr2:72933595-72933617
ctgccatccccttctgtgaatgt

SEQ ID NO: 123 - DNA, 22 bp, Homo sapiens, chr2:72934372-72934393
ggaatctaccaccccaggctct

SEQ ID NO: 124 - DNA, 23 bp, Homo sapiens, chr6:43770819-43770841
gaccccctccaccccgcctccgg

SEQ ID NO: 125 - DNA, 20 bp, Homo sapiens, chr6:43770305-43770324
tcagcggactcaccggccag

SEQ ID NO: 126 - DNA, 20 bp, Homo sapiens, chr6:43771025-43771044
gcgccgagtcgccactgcgg

SEQ ID NO: 127 - DNA, 23 bp, Homo sapiens, chr11:22625792-22625814
gctgcagaagggattccatgagg

SEQ ID NO: 128 - DNA, 21 bp, Homo sapiens, chr11:22625410-22625430
gccaggctctcttggagtgtc

SEQ ID NO: 129 - DNA, 24 bp, Homo sapiens, chr11:22626287-22626310
agcatagcgcctggcattaatagg

SEQ ID NO: 130 - DNA, 23 bp, Homo sapiens, chr22:36556948-36556970
gctgcagaagggattccaagagg

SEQ ID NO: 131 - DNA, 24 bp, Homo sapiens, chr22:36556738-36556761
cccgtgaggtgctgagatttgaac

SEQ ID NO: 132 - DNA, 21 bp, Homo sapiens, chr22:36557440-36557460
cacatggaggaggtgacgctg

SEQ ID NO: 133 - DNA, 23 bp, Homo sapiens, chr3:46373262-46373284
ggtacctatcgattgtcaggagg

SEQ ID NO: 134 - DNA, 24 bp, Homo sapiens, chr3:46372884-46372907
atgcacagggtggaacaagatgga

SEQ ID NO: 135 - DNA, 24 bp, Homo sapiens, chr3:46373989-46374012
ctaagccatgtgcacaactctgac

SEQ ID NO: 136 - DNA, 23 bp, Homo sapiens, chr3:46357923-46357945
ggtatctatcgattgtcaggagg

SEQ ID NO: 137 - DNA, 23 bp, Homo sapiens, chr3:46357814-46357836
cattgtgggctcactctgctgca

SEQ ID NO: 138 - DNA, 25 bp, Homo sapiens, chr3:46358817-46358841
ctgagatgagctttctggagagtca